European Patent Application EP 4 756 027 A1, published June 10, 2026. Title: DOUBLE-STRANDED RIBONUCLEIC ACID TARGETING PD-L1. Applicant: Chia Tai Tianqing Pharmaceutical Group Co., Ltd. The sequence listing filed with the application follows.

SEQUENCE LISTING (58 sequences)

SEQ ID NO: 1 - DNA, 21 bp, synthetic construct
  source 1..21: mol_type = other DNA; note; note (original language) = Human PD-L1 primer
tggcatttgctgaacgcattt

SEQ ID NO: 2 - DNA, 22 bp, synthetic construct
  source 1..22: mol_type = other DNA; note; note (original language) = Human PD-L1 primer
tgcagccaggtctaattgtttt

SEQ ID NO: 3 - DNA, 20 bp, synthetic construct
  source 1..20: mol_type = other DNA; note; note (original language) = Human PD-L1 primer
tggctcccagaattaccaag

SEQ ID NO: 4 - DNA, 20 bp, synthetic construct
  source 1..20: mol_type = other DNA; note; note (original language) = Human PD-L1 primer
tatggtggtgccgactacaa

SEQ ID NO: 5 - DNA, 20 bp, synthetic construct
  source 1..20: mol_type = other DNA; note; note (original language) = Mouse PD-L1 primer
ccgggatgagagatggagtc

SEQ ID NO: 6 - DNA, 21 bp, synthetic construct
  source 1..21: mol_type = other DNA; note; note (original language) = Mouse PD-L1 primer
tgtcgtcagaattcaccagtc

SEQ ID NO: 7 - DNA, 20 bp, synthetic construct
  source 1..20: mol_type = other DNA; note; note (original language) = Mouse GAPDH primer
atgaaggggtcgttgatggc

SEQ ID NO: 8 - DNA, 23 bp, synthetic construct
  source 1..23: mol_type = other DNA; note; note (original language) = Mouse GAPDH primer
gggttcctataaatacggactgc

SEQ ID NO: 9 - RNA, 21 nt, synthetic construct
  source 1..21: mol_type = other RNA; note; note (original language) = Sense strand
agcaatatgacaattgaatga

SEQ ID NO: 10 - RNA, 23 nt, synthetic construct
  source 1..23: mol_type = other RNA; note; note (original language) = Antisense strand
tcattcaattgtcatattgctac

SEQ ID NO: 11 - RNA, 21 nt, synthetic construct
  source 1..21: mol_type = other RNA; note; note (original language) = Sense strand
atttactgtcacggttcccaa

SEQ ID NO: 12 - RNA, 23 nt, synthetic construct
  source 1..23: mol_type = other RNA; note; note (original language) = Antisense strand
ttgggaaccgtgacagtaatagc

SEQ ID NO: 13 - RNA, 19 nt, synthetic construct
  source 1..19: mol_type = other RNA; note; note (original language) = Sense strand
ctatttattttgagtctgt

SEQ ID NO: 14 - RNA, 21 nt, synthetic construct
  source 1..21: mol_type = other RNA; note; note (original language) = Antisense strand
acagactcaaaataaatagga

SEQ ID NO: 15 - RNA, 21 nt, synthetic construct
  source 1..21: mol_type = other RNA; note; note (original language) = Sense strand
tgaagatatattgtagtagat

SEQ ID NO: 16 - RNA, 23 nt, synthetic construct
  source 1..23: mol_type = other RNA; note; note (original language) = Antisense strand
atctactacaatatatcttcaaa

SEQ ID NO: 17 - RNA, 21 nt, synthetic construct
  source 1..21: mol_type = other RNA; note; note (original language) = Sense strand
ttgtctcatgtttcatcgtaa

SEQ ID NO: 18 - RNA, 23 nt, synthetic construct
  source 1..23: mol_type = other RNA; note; note (original language) = Antisense strand
ttacgatgaaacatgagacaaaa

SEQ ID NO: 19 - RNA, 21 nt, synthetic construct
  source 1..21: mol_type = other RNA; note; note (original language) = Sense strand
ctgtgcagtatctgttccatt

SEQ ID NO: 20 - RNA, 23 nt, synthetic construct
  source 1..23: mol_type = other RNA; note; note (original language) = Antisense strand
aatggaacagatactgcacagac

SEQ ID NO: 21 - RNA, 21 nt, synthetic construct
  source 1..21: mol_type = other RNA; note; note (original language) = Sense strand
aatgaaaggactcacttggta

SEQ ID NO: 22 - RNA, 23 nt, synthetic construct
  source 1..23: mol_type = other RNA; note; note (original language) = Antisense strand
taccaagtgagtcctttcatttg

SEQ ID NO: 23 - RNA, 21 nt, synthetic construct
  source 1..21: mol_type = other RNA; note; note (original language) = Sense strand
gctgcatgatcagctatggta

SEQ ID NO: 24 - RNA, 23 nt, synthetic construct
  source 1..23: mol_type = other RNA; note; note (original language) = Antisense strand
taccatagctgatcatgcagcgg

SEQ ID NO: 25 - RNA, 21 nt, synthetic construct
  source 1..21: mol_type = other RNA; note; note (original language) = Sense strand
ggtgcttggtctcctctataa

SEQ ID NO: 26 - RNA, 23 nt, synthetic construct
  source 1..23: mol_type = other RNA; note; note (original language) = Antisense strand
ttatagaggagaccaagcacctt

SEQ ID NO: 27 - RNA, 21 nt, synthetic construct
  source 1..21: mol_type = other RNA; note; note (original language) = Sense strand
attggtcatcccagaactaca

SEQ ID NO: 28 - RNA, 23 nt, synthetic construct
  source 1..23: mol_type = other RNA; note; note (original language) = Antisense strand
tgtagttctgggatgaccaattc

SEQ ID NO: 29 - RNA, 19 nt, synthetic construct
  source 1..19: mol_type = other RNA; note; note (original language) = Sense strand
tatttattttgagtctgtg

SEQ ID NO: 30 - RNA, 21 nt, synthetic construct
  source 1..21: mol_type = other RNA; note; note (original language) = Antisense strand
cacagactcaaaataaatagg

SEQ ID NO: 31 - RNA, 21 nt, synthetic construct
  source 1..21: mol_type = other RNA; note; note (original language) = Sense strand
  modified_base 1..8: mod_base = OTHER; note; note (original language) = 2'-O-methyl modification
  modified_base 9..11: mod_base = OTHER; note; note (original language) = 2'-fluoro modification
  modified_base 12..21: mod_base = OTHER; note; note (original language) = 2'-O-methyl modification
  modified_base 1^2: mod_base = OTHER; note; note (original language) = Phosphorothioate linkage
  modified_base 2^3: mod_base = OTHER; note; note (original language) = Phosphorothioate linkage
agcaatatgacaattgaatga

SEQ ID NO: 32 - RNA, 23 nt, synthetic construct
  source 1..23: mol_type = other RNA; note; note (original language) = Antisense strand
  modified_base 1: mod_base = OTHER; note; note (original language) = 2'-O-methyl modification
  modified_base 2: mod_base = OTHER; note; note (original language) = 2'-fluoro modification
  modified_base 3..5: mod_base = OTHER; note; note (original language) = 2'-O-methyl modification
  modified_base 6: mod_base = OTHER; note; note (original language) = 2'-fluoro modification
  modified_base 7..13: mod_base = OTHER; note; note (original language) = 2'-O-methyl modification
  modified_base 14: mod_base = OTHER; note; note (original language) = 2'-fluoro modification
  modified_base 15: mod_base = OTHER; note; note (original language) = 2'-O-methyl modification
  modified_base 16: mod_base = OTHER; note; note (original language) = 2'-fluoro modification
  modified_base 17..23: mod_base = OTHER; note; note (original language) = 2'-O-methyl modification
  modified_base 1^2: mod_base = OTHER; note; note (original language) = Phosphorothioate linkage
  modified_base 2^3: mod_base = OTHER; note; note (original language) = Phosphorothioate linkage
  modified_base 21^22: mod_base = OTHER; note; note (original language) = Phosphorothioate linkage
  modified_base 22^23: mod_base = OTHER; note; note (original language) = Phosphorothioate linkage
tcattcaattgtcatattgctac

SEQ ID NO: 33 - RNA, 21 nt, synthetic construct
  source 1..21: mol_type = other RNA; note; note (original language) = Sense strand
  modified_base 1..8: mod_base = OTHER; note; note (original language) = 2'-O-methyl modification
  modified_base 9..11: mod_base = OTHER; note; note (original language) = 2'-fluoro modification
  modified_base 12..21: mod_base = OTHER; note; note (original language) = 2'-O-methyl modification
  modified_base 1^2: mod_base = OTHER; note; note (original language) = Phosphorothioate linkage
  modified_base 2^3: mod_base = OTHER; note; note (original language) = Phosphorothioate linkage
atttactgtcacggttcccaa

SEQ ID NO: 34 - RNA, 23 nt, synthetic construct
  source 1..23: mol_type = other RNA; note; note (original language) = Antisense strand
  modified_base 1: mod_base = OTHER; note; note (original language) = 2'-O-methyl modification
  modified_base 2: mod_base = OTHER; note; note (original language) = 2'-fluoro modification
  modified_base 3..5: mod_base = OTHER; note; note (original language) = 2'-O-methyl modification
  modified_base 6: mod_base = OTHER; note; note (original language) = 2'-fluoro modification
  modified_base 7..13: mod_base = OTHER; note; note (original language) = 2'-O-methyl modification
  modified_base 14: mod_base = OTHER; note; note (original language) = 2'-fluoro modification
  modified_base 15: mod_base = OTHER; note; note (original language) = 2'-O-methyl modification
  modified_base 16: mod_base = OTHER; note; note (original language) = 2'-fluoro modification
  modified_base 17..23: mod_base = OTHER; note; note (original language) = 2'-O-methyl modification
  modified_base 1^2: mod_base = OTHER; note; note (original language) = Phosphorothioate linkage
  modified_base 2^3: mod_base = OTHER; note; note (original language) = Phosphorothioate linkage
  modified_base 21^22: mod_base = OTHER; note; note (original language) = Phosphorothioate linkage
  modified_base 22^23: mod_base = OTHER; note; note (original language) = Phosphorothioate linkage
ttgggaaccgtgacagtaatagc

SEQ ID NO: 35 - RNA, 19 nt, synthetic construct
  source 1..19: mol_type = other RNA; note; note (original language) = Sense strand
  modified_base 1..6: mod_base = OTHER; note; note (original language) = 2'-O-methyl modification
  modified_base 7..9: mod_base = OTHER; note; note (original language) = 2'-fluoro modification
  modified_base 10..19: mod_base = OTHER; note; note (original language) = 2'-O-methyl modification
  modified_base 1^2: mod_base = OTHER; note; note (original language) = Phosphorothioate linkage
  modified_base 2^3: mod_base = OTHER; note; note (original language) = Phosphorothioate linkage
ctatttattttgagtctgt

SEQ ID NO: 36 - RNA, 21 nt, synthetic construct
  source 1..21: mol_type = other RNA; note; note (original language) = Antisense strand
  modified_base 1: mod_base = OTHER; note; note (original language) = 2'-O-methyl modification
  modified_base 2: mod_base = OTHER; note; note (original language) = 2'-fluoro modification
  modified_base 3..5: mod_base = OTHER; note; note (original language) = 2'-O-methyl modification
  modified_base 6: mod_base = OTHER; note; note (original language) = 2'-fluoro modification
  modified_base 7..13: mod_base = OTHER; note; note (original language) = 2'-O-methyl modification
  modified_base 14: mod_base = OTHER; note; note (original language) = 2'-fluoro modification
  modified_base 15: mod_base = OTHER; note; note (original language) = 2'-O-methyl modification
  modified_base 16: mod_base = OTHER; note; note (original language) = 2'-fluoro modification
  modified_base 17..21: mod_base = OTHER; note; note (original language) = 2'-O-methyl modification
  modified_base 1^2: mod_base = OTHER; note; note (original language) = Phosphorothioate linkage
  modified_base 2^3: mod_base = OTHER; note; note (original language) = Phosphorothioate linkage
  modified_base 19^20: mod_base = OTHER; note; note (original language) = Phosphorothioate linkage
  modified_base 20^21: mod_base = OTHER; note; note (original language) = Phosphorothioate linkage
acagactcaaaataaatagga

SEQ ID NO: 37 - RNA, 21 nt, synthetic construct
  source 1..21: mol_type = other RNA; note; note (original language) = Sense strand
  modified_base 1..8: mod_base = OTHER; note; note (original language) = 2'-O-methyl modification
  modified_base 9..11: mod_base = OTHER; note; note (original language) = 2'-fluoro modification
  modified_base 12..21: mod_base = OTHER; note; note (original language) = 2'-O-methyl modification
  modified_base 1^2: mod_base = OTHER; note; note (original language) = Phosphorothioate linkage
  modified_base 2^3: mod_base = OTHER; note; note (original language) = Phosphorothioate linkage
tgaagatatattgtagtagat

SEQ ID NO: 38 - RNA, 23 nt, synthetic construct
  source 1..23: mol_type = other RNA; note; note (original language) = Antisense strand
  modified_base 1: mod_base = OTHER; note; note (original language) = 2'-O-methyl modification
  modified_base 2: mod_base = OTHER; note; note (original language) = 2'-fluoro modification
  modified_base 3..5: mod_base = OTHER; note; note (original language) = 2'-O-methyl modification
  modified_base 6: mod_base = OTHER; note; note (original language) = 2'-fluoro modification
  modified_base 7..13: mod_base = OTHER; note; note (original language) = 2'-O-methyl modification
  modified_base 14: mod_base = OTHER; note; note (original language) = 2'-fluoro modification
  modified_base 15: mod_base = OTHER; note; note (original language) = 2'-O-methyl modification
  modified_base 16: mod_base = OTHER; note; note (original language) = 2'-fluoro modification
  modified_base 17..23: mod_base = OTHER; note; note (original language) = 2'-O-methyl modification
  modified_base 1^2: mod_base = OTHER; note; note (original language) = Phosphorothioate linkage
  modified_base 2^3: mod_base = OTHER; note; note (original language) = Phosphorothioate linkage
  modified_base 21^22: mod_base = OTHER; note; note (original language) = Phosphorothioate linkage
  modified_base 22^23: mod_base = OTHER; note; note (original language) = Phosphorothioate linkage
atctactacaatatatcttcaaa

SEQ ID NO: 39 - RNA, 21 nt, synthetic construct
  source 1..21: mol_type = other RNA; note; note (original language) = Sense strand
  modified_base 1..8: mod_base = OTHER; note; note (original language) = 2'-O-methyl modification
  modified_base 9..11: mod_base = OTHER; note; note (original language) = 2'-fluoro modification
  modified_base 12..21: mod_base = OTHER; note; note (original language) = 2'-O-methyl modification
  modified_base 1^2: mod_base = OTHER; note; note (original language) = Phosphorothioate linkage
  modified_base 2^3: mod_base = OTHER; note; note (original language) = Phosphorothioate linkage
ttgtctcatgtttcatcgtaa

SEQ ID NO: 40 - RNA, 23 nt, synthetic construct
  source 1..23: mol_type = other RNA; note; note (original language) = Antisense strand
  modified_base 1: mod_base = OTHER; note; note (original language) = 2'-O-methyl modification
  modified_base 2: mod_base = OTHER; note; note (original language) = 2'-fluoro modification
  modified_base 3..5: mod_base = OTHER; note; note (original language) = 2'-O-methyl modification
  modified_base 6: mod_base = OTHER; note; note (original language) = 2'-fluoro modification
  modified_base 7..13: mod_base = OTHER; note; note (original language) = 2'-O-methyl modification
  modified_base 14: mod_base = OTHER; note; note (original language) = 2'-fluoro modification
  modified_base 15: mod_base = OTHER; note; note (original language) = 2'-O-methyl modification
  modified_base 16: mod_base = OTHER; note; note (original language) = 2'-fluoro modification
  modified_base 17..23: mod_base = OTHER; note; note (original language) = 2'-O-methyl modification
  modified_base 1^2: mod_base = OTHER; note; note (original language) = Phosphorothioate linkage
  modified_base 2^3: mod_base = OTHER; note; note (original language) = Phosphorothioate linkage
  modified_base 21^22: mod_base = OTHER; note; note (original language) = Phosphorothioate linkage
  modified_base 22^23: mod_base = OTHER; note; note (original language) = Phosphorothioate linkage
ttacgatgaaacatgagacaaaa

SEQ ID NO: 41 - RNA, 21 nt, synthetic construct
  source 1..21: mol_type = other RNA; note; note (original language) = Sense strand
  modified_base 1..8: mod_base = OTHER; note; note (original language) = 2'-O-methyl modification
  modified_base 9..11: mod_base = OTHER; note; note (original language) = 2'-fluoro modification
  modified_base 12..21: mod_base = OTHER; note; note (original language) = 2'-O-methyl modification
  modified_base 1^2: mod_base = OTHER; note; note (original language) = Phosphorothioate linkage
  modified_base 2^3: mod_base = OTHER; note; note (original language) = Phosphorothioate linkage
ctgtgcagtatctgttccatt

SEQ ID NO: 42 - RNA, 23 nt, synthetic construct
  source 1..23: mol_type = other RNA; note; note (original language) = Antisense strand
  modified_base 1: mod_base = OTHER; note; note (original language) = 2'-O-methyl modification
  modified_base 2: mod_base = OTHER; note; note (original language) = 2'-fluoro modification
  modified_base 3..5: mod_base = OTHER; note; note (original language) = 2'-O-methyl modification
  modified_base 6: mod_base = OTHER; note; note (original language) = 2'-fluoro modification
  modified_base 7..13: mod_base = OTHER; note; note (original language) = 2'-O-methyl modification
  modified_base 14: mod_base = OTHER; note; note (original language) = 2'-fluoro modification
  modified_base 15: mod_base = OTHER; note; note (original language) = 2'-O-methyl modification
  modified_base 16: mod_base = OTHER; note; note (original language) = 2'-fluoro modification
  modified_base 17..23: mod_base = OTHER; note; note (original language) = 2'-O-methyl modification
  modified_base 1^2: mod_base = OTHER; note; note (original language) = Phosphorothioate linkage
  modified_base 2^3: mod_base = OTHER; note; note (original language) = Phosphorothioate linkage
  modified_base 21^22: mod_base = OTHER; note; note (original language) = Phosphorothioate linkage
  modified_base 22^23: mod_base = OTHER; note; note (original language) = Phosphorothioate linkage
aatggaacagatactgcacagac

SEQ ID NO: 43 - RNA, 21 nt, synthetic construct
  source 1..21: mol_type = other RNA; note; note (original language) = Sense strand
  modified_base 1..8: mod_base = OTHER; note; note (original language) = 2'-O-methyl modification
  modified_base 9..11: mod_base = OTHER; note; note (original language) = 2'-fluoro modification
  modified_base 12..21: mod_base = OTHER; note; note (original language) = 2'-O-methyl modification
  modified_base 1^2: mod_base = OTHER; note; note (original language) = Phosphorothioate linkage
  modified_base 2^3: mod_base = OTHER; note; note (original language) = Phosphorothioate linkage
aatgaaaggactcacttggta

SEQ ID NO: 44 - RNA, 23 nt, synthetic construct
  source 1..23: mol_type = other RNA; note; note (original language) = Antisense strand
  modified_base 1: mod_base = OTHER; note; note (original language) = 2'-O-methyl modification
  modified_base 2: mod_base = OTHER; note; note (original language) = 2'-fluoro modification
  modified_base 3..5: mod_base = OTHER; note; note (original language) = 2'-O-methyl modification
  modified_base 6: mod_base = OTHER; note; note (original language) = 2'-fluoro modification
  modified_base 7..13: mod_base = OTHER; note; note (original language) = 2'-O-methyl modification
  modified_base 14: mod_base = OTHER; note; note (original language) = 2'-fluoro modification
  modified_base 15: mod_base = OTHER; note; note (original language) = 2'-O-methyl modification
  modified_base 16: mod_base = OTHER; note; note (original language) = 2'-fluoro modification
  modified_base 17..23: mod_base = OTHER; note; note (original language) = 2'-O-methyl modification
  modified_base 1^2: mod_base = OTHER; note; note (original language) = Phosphorothioate linkage
  modified_base 2^3: mod_base = OTHER; note; note (original language) = Phosphorothioate linkage
  modified_base 21^22: mod_base = OTHER; note; note (original language) = Phosphorothioate linkage
  modified_base 22^23: mod_base = OTHER; note; note (original language) = Phosphorothioate linkage
taccaagtgagtcctttcatttg

SEQ ID NO: 45 - RNA, 21 nt, synthetic construct
  source 1..21: mol_type = other RNA; note; note (original language) = Sense strand
  modified_base 1..8: mod_base = OTHER; note; note (original language) = 2'-O-methyl modification
  modified_base 9..11: mod_base = OTHER; note; note (original language) = 2'-fluoro modification
  modified_base 12..21: mod_base = OTHER; note; note (original language) = 2'-O-methyl modification
  modified_base 1^2: mod_base = OTHER; note; note (original language) = Phosphorothioate linkage
  modified_base 2^3: mod_base = OTHER; note; note (original language) = Phosphorothioate linkage
gctgcatgatcagctatggta

SEQ ID NO: 46 - RNA, 23 nt, synthetic construct
  source 1..23: mol_type = other RNA; note; note (original language) = Antisense strand
  modified_base 1: mod_base = OTHER; note; note (original language) = 2'-O-methyl modification
  modified_base 2: mod_base = OTHER; note; note (original language) = 2'-fluoro modification
  modified_base 3..5: mod_base = OTHER; note; note (original language) = 2'-O-methyl modification
  modified_base 6: mod_base = OTHER; note; note (original language) = 2'-fluoro modification
  modified_base 7..13: mod_base = OTHER; note; note (original language) = 2'-O-methyl modification
  modified_base 14: mod_base = OTHER; note; note (original language) = 2'-fluoro modification
  modified_base 15: mod_base = OTHER; note; note (original language) = 2'-O-methyl modification
  modified_base 16: mod_base = OTHER; note; note (original language) = 2'-fluoro modification
  modified_base 17..23: mod_base = OTHER; note; note (original language) = 2'-O-methyl modification
  modified_base 1^2: mod_base = OTHER; note; note (original language) = Phosphorothioate linkage
  modified_base 2^3: mod_base = OTHER; note; note (original language) = Phosphorothioate linkage
  modified_base 21^22: mod_base = OTHER; note; note (original language) = Phosphorothioate linkage
  modified_base 22^23: mod_base = OTHER; note; note (original language) = Phosphorothioate linkage
taccatagctgatcatgcagcgg

SEQ ID NO: 47 - RNA, 21 nt, synthetic construct
  source 1..21: mol_type = other RNA; note; note (original language) = Sense strand
  modified_base 1..8: mod_base = OTHER; note; note (original language) = 2'-O-methyl modification
  modified_base 9..11: mod_base = OTHER; note; note (original language) = 2'-fluoro modification
  modified_base 12..21: mod_base = OTHER; note; note (original language) = 2'-O-methyl modification
  modified_base 1^2: mod_base = OTHER; note; note (original language) = Phosphorothioate linkage
  modified_base 2^3: mod_base = OTHER; note; note (original language) = Phosphorothioate linkage
ggtgcttggtctcctctataa

SEQ ID NO: 48 - RNA, 23 nt, synthetic construct
  source 1..23: mol_type = other RNA; note; note (original language) = Antisense strand
  modified_base 1: mod_base = OTHER; note; note (original language) = 2'-O-methyl modification
  modified_base 2: mod_base = OTHER; note; note (original language) = 2'-fluoro modification
  modified_base 3..5: mod_base = OTHER; note; note (original language) = 2'-O-methyl modification
  modified_base 6: mod_base = OTHER; note; note (original language) = 2'-fluoro modification
  modified_base 7..13: mod_base = OTHER; note; note (original language) = 2'-O-methyl modification
  modified_base 14: mod_base = OTHER; note; note (original language) = 2'-fluoro modification
  modified_base 15: mod_base = OTHER; note; note (original language) = 2'-O-methyl modification
  modified_base 16: mod_base = OTHER; note; note (original language) = 2'-fluoro modification
  modified_base 17..23: mod_base = OTHER; note; note (original language) = 2'-O-methyl modification
  modified_base 1^2: mod_base = OTHER; note; note (original language) = Phosphorothioate linkage
  modified_base 2^3: mod_base = OTHER; note; note (original language) = Phosphorothioate linkage
  modified_base 21^22: mod_base = OTHER; note; note (original language) = Phosphorothioate linkage
  modified_base 22^23: mod_base = OTHER; note; note (original language) = Phosphorothioate linkage
ttatagaggagaccaagcacctt

SEQ ID NO: 49 - RNA, 21 nt, synthetic construct
  source 1..21: mol_type = other RNA; note; note (original language) = Sense strand
  modified_base 1..8: mod_base = OTHER; note; note (original language) = 2'-O-methyl modification
  modified_base 9..11: mod_base = OTHER; note; note (original language) = 2'-fluoro modification
  modified_base 12..21: mod_base = OTHER; note; note (original language) = 2'-O-methyl modification
  modified_base 1^2: mod_base = OTHER; note; note (original language) = Phosphorothioate linkage
  modified_base 2^3: mod_base = OTHER; note; note (original language) = Phosphorothioate linkage
attggtcatcccagaactaca

SEQ ID NO: 50 - RNA, 23 nt, synthetic construct
  source 1..23: mol_type = other RNA; note; note (original language) = Antisense strand
  modified_base 1: mod_base = OTHER; note; note (original language) = 2'-O-methyl modification
  modified_base 2: mod_base = OTHER; note; note (original language) = 2'-fluoro modification
  modified_base 3..5: mod_base = OTHER; note; note (original language) = 2'-O-methyl modification
  modified_base 6: mod_base = OTHER; note; note (original language) = 2'-fluoro modification
  modified_base 7..13: mod_base = OTHER; note; note (original language) = 2'-O-methyl modification
  modified_base 14: mod_base = OTHER; note; note (original language) = 2'-fluoro modification
  modified_base 15: mod_base = OTHER; note; note (original language) = 2'-O-methyl modification
  modified_base 16: mod_base = OTHER; note; note (original language) = 2'-fluoro modification
  modified_base 17..23: mod_base = OTHER; note; note (original language) = 2'-O-methyl modification
  modified_base 1^2: mod_base = OTHER; note; note (original language) = Phosphorothioate linkage
  modified_base 2^3: mod_base = OTHER; note; note (original language) = Phosphorothioate linkage
  modified_base 21^22: mod_base = OTHER; note; note (original language) = Phosphorothioate linkage
  modified_base 22^23: mod_base = OTHER; note; note (original language) = Phosphorothioate linkage
tgtagttctgggatgaccaattc

SEQ ID NO: 51 - RNA, 19 nt, synthetic construct
  source 1..19: mol_type = other RNA; note; note (original language) = Sense strand
  modified_base 1..6: mod_base = OTHER; note; note (original language) = 2'-O-methyl modification
  modified_base 7..9: mod_base = OTHER; note; note (original language) = 2'-fluoro modification
  modified_base 10..19: mod_base = OTHER; note; note (original language) = 2'-O-methyl modification
  modified_base 1^2: mod_base = OTHER; note; note (original language) = Phosphorothioate linkage
  modified_base 2^3: mod_base = OTHER; note; note (original language) = Phosphorothioate linkage
tatttattttgagtctgtg

SEQ ID NO: 52 - RNA, 21 nt, synthetic construct
  source 1..21: mol_type = other RNA; note; note (original language) = Antisense strand
  modified_base 1: mod_base = OTHER; note; note (original language) = 2'-O-methyl modification
  modified_base 2: mod_base = OTHER; note; note (original language) = 2'-fluoro modification
  modified_base 3..5: mod_base = OTHER; note; note (original language) = 2'-O-methyl modification
  modified_base 6: mod_base = OTHER; note; note (original language) = 2'-fluoro modification
  modified_base 7..13: mod_base = OTHER; note; note (original language) = 2'-O-methyl modification
  modified_base 14: mod_base = OTHER; note; note (original language) = 2'-fluoro modification
  modified_base 15: mod_base = OTHER; note; note (original language) = 2'-O-methyl modification
  modified_base 16: mod_base = OTHER; note; note (original language) = 2'-fluoro modification
  modified_base 17..21: mod_base = OTHER; note; note (original language) = 2'-O-methyl modification
  modified_base 1^2: mod_base = OTHER; note; note (original language) = Phosphorothioate linkage
  modified_base 2^3: mod_base = OTHER; note; note (original language) = Phosphorothioate linkage
  modified_base 19^20: mod_base = OTHER; note; note (original language) = Phosphorothioate linkage
  modified_base 20^21: mod_base = OTHER; note; note (original language) = Phosphorothioate linkage
cacagactcaaaataaatagg

SEQ ID NO: 53 - RNA, 21 nt, synthetic construct
  source 1..21: mol_type = other RNA; note; note (original language) = Sense strand
atttactgtcacggttcccaa

SEQ ID NO: 54 - RNA, 23 nt, synthetic construct
  source 1..23: mol_type = other RNA; note; note (original language) = Antisense strand
ttgggaaccgtgacagtaaatgc

SEQ ID NO: 55 - RNA, 21 nt, synthetic construct
  source 1..21: mol_type = other RNA; note; note (original language) = Sense strand
  modified_base 1..8: mod_base = OTHER; note; note (original language) = 2'-O-methyl modification
  modified_base 9..11: mod_base = OTHER; note; note (original language) = 2'-fluoro modification
  modified_base 12..21: mod_base = OTHER; note; note (original language) = 2'-O-methyl modification
  modified_base 1^2: mod_base = OTHER; note; note (original language) = Phosphorothioate linkage
  modified_base 2^3: mod_base = OTHER; note; note (original language) = Phosphorothioate linkage
atttactgtcacggttcccaa

SEQ ID NO: 56 - RNA, 23 nt, synthetic construct
  source 1..23: mol_type = other RNA; note; note (original language) = Antisense strand
  modified_base 1: mod_base = OTHER; note; note (original language) = 2'-O-methyl modification
  modified_base 2: mod_base = OTHER; note; note (original language) = 2'-fluoro modification
  modified_base 3..5: mod_base = OTHER; note; note (original language) = 2'-O-methyl modification
  modified_base 6: mod_base = OTHER; note; note (original language) = 2'-fluoro modification
  modified_base 7..13: mod_base = OTHER; note; note (original language) = 2'-O-methyl modification
  modified_base 14: mod_base = OTHER; note; note (original language) = 2'-fluoro modification
  modified_base 15: mod_base = OTHER; note; note (original language) = 2'-O-methyl modification
  modified_base 16: mod_base = OTHER; note; note (original language) = 2'-fluoro modification
  modified_base 17..23: mod_base = OTHER; note; note (original language) = 2'-O-methyl modification
  modified_base 1^2: mod_base = OTHER; note; note (original language) = Phosphorothioate linkage
  modified_base 2^3: mod_base = OTHER; note; note (original language) = Phosphorothioate linkage
  modified_base 21^22: mod_base = OTHER; note; note (original language) = Phosphorothioate linkage
  modified_base 22^23: mod_base = OTHER; note; note (original language) = Phosphorothioate linkage
ttgggaaccgtgacagtaaatgc

SEQ ID NO: 57 - DNA, 19 bp, synthetic construct
  source 1..19: mol_type = other DNA; note; note (original language) = Human GAPDH primer
ggtcggagtcaacggattt

SEQ ID NO: 58 - DNA, 19 bp, synthetic construct
  source 1..19: mol_type = other DNA; note; note (original language) = Human GAPDH primer
ccagcatcgccccacttga